European Patent Application EP 4 541 814 A1, published April 23, 2025. Title: Stabilized polypeptides. Applicant: Cytiva BioProcess R&D AB. The sequence listing filed with the application follows.

SEQUENCE LISTING (195 sequences)

SEQ ID NO: 1 - protein, 26 aa, synthetic construct
  VARIANT 1: note = X is Q or V or E or D
  VARIANT 2: note = X is V or D
  VARIANT 5: note = X is Q or V or E
  VARIANT 11: note = X is S or L
  VARIANT 14: note = X is A or S or T
  VARIANT 19: note = X is R or S or K or T
  VARIANT 23: note = X is T or V or A or S
  VARIANT 24: note = X is I or V or S
XXQLXZSGGGXVQXGGSLXLSCXXSG

SEQ ID NO: 2 - protein, 14 aa, synthetic construct
  VARIANT 5: note = X is R or I or T or K
  VARIANT 8: note = X is R or K or Q or G or E
  VARIANT 9: note = X is E or Q or A or D or G
  VARIANT 10: note = X is R or I or L
  VARIANT 12: note = X is F or L
WFRQXPGXXXEXVA

SEQ ID NO: 3 - protein, 39 aa, synthetic construct
  VARIANT 2: note = X is A or T or N or Q or S
  VARIANT 3: note = X is D or S
  VARIANT 4: note = X is S or A
  VARIANT 6: note = X is K or A
  VARIANT 18: note = X is N or Q
  VARIANT 20: note = X is V or A
  VARIANT 21: note = X is Y or A or W or F
  VARIANT 26: note = X is N or S or T or Q
  VARIANT 34: note = X is V or I or L or A
YXXXVXGRFTISRDNAKXTXXLQMNXLKPEDTAXYYCAA

SEQ ID NO: 4 - protein, 26 aa, synthetic construct
QVQLQESGGGSVQAGGSLRLSCVASG

SEQ ID NO: 5 - protein, 26 aa, synthetic construct
QVQLQESGGGSVQAGGSLTLSCVASG

SEQ ID NO: 6 - protein, 26 aa, synthetic construct
QVQLQESGGGSVQAGGSLRLSCTASG

SEQ ID NO: 7 - protein, 26 aa, synthetic construct
QVQLQESGGGSVQAGGSLTLSCTASG

SEQ ID NO: 8 - protein, 26 aa, synthetic construct
QVQLQQSGGGSVQAGGSLRLSCTISG

SEQ ID NO: 9 - protein, 26 aa, synthetic construct
QVQLQESGGGSVQAGGSLRLSCTISG

SEQ ID NO: 10 - protein, 26 aa, synthetic construct
QVQLQQSGGGSVQAGGSLRLSCTVSG

SEQ ID NO: 11 - protein, 26 aa, synthetic construct
QVQLQQSGGGSVQAGGSLTLSCTISG

SEQ ID NO: 12 - protein, 26 aa, synthetic construct
QVQLVQSGGGSVQAGGSLRLSCTISG

SEQ ID NO: 13 - protein, 26 aa, synthetic construct
QVQLEQSGGGSVQAGGSLRLSCTISG

SEQ ID NO: 14 - protein, 26 aa, synthetic construct
QVQLQQSGGGSVQSGGSLRLSCTISG

SEQ ID NO: 15 - protein, 26 aa, synthetic construct
QVQLQQSGGGSVQTGGSLRLSCTISG

SEQ ID NO: 16 - protein, 26 aa, synthetic construct
QVQLQQSGGGSVQAGGSLKLSCTISG

SEQ ID NO: 17 - protein, 26 aa, synthetic construct
QVQLQQSGGGSVQAGGSLSLSCTISG

SEQ ID NO: 18 - protein, 26 aa, synthetic construct
QVQLQQSGGGSVQAGGSLRLSCVISG

SEQ ID NO: 19 - protein, 26 aa, synthetic construct
QVQLQQSGGGSVQAGGSLRLSCSISG

SEQ ID NO: 20 - protein, 26 aa, synthetic construct
QVQLQQSGGGSVQAGGSLRLSCAISG

SEQ ID NO: 21 - protein, 26 aa, synthetic construct
QVQLQQSGGGSVQAGGSLRLSCTSSG

SEQ ID NO: 22 - protein, 26 aa, synthetic construct
QVQLVESGGGSVQAGGSLSLSCTISG

SEQ ID NO: 23 - protein, 14 aa, synthetic construct
WFRQPPGKAREFVA

SEQ ID NO: 24 - protein, 14 aa, synthetic construct
WFRQRPGKAREFVA

SEQ ID NO: 25 - skipped

SEQ ID NO: 26 - protein, 14 aa, synthetic construct
WFRQRPGKEREFVA

SEQ ID NO: 27 - protein, 14 aa, synthetic construct
WFRQPPGKEREFVA

SEQ ID NO: 28 - protein, 14 aa, synthetic construct
WFRQTPGKEREFVA

SEQ ID NO: 29 - protein, 14 aa, synthetic construct
WFRQIPGKEREFVA

SEQ ID NO: 30 - protein, 14 aa, synthetic construct
WFRQKPGKEREFVA

SEQ ID NO: 31 - protein, 14 aa, synthetic construct
WFRQAPGKEREFVA

SEQ ID NO: 32 - protein, 14 aa, synthetic construct
WFRQRPGGEREFVA

SEQ ID NO: 33 - protein, 14 aa, synthetic construct
WFRQRPGQEREFVA

SEQ ID NO: 34 - protein, 14 aa, synthetic construct
WFRQRPGREREFVA

SEQ ID NO: 35 - protein, 14 aa, synthetic construct
WFRQRPGKQREFVA

SEQ ID NO: 36 - protein, 14 aa, synthetic construct
WFRQRPGKDREFVA

SEQ ID NO: 37 - protein, 14 aa, synthetic construct
WFRQRPGKGREFVA

SEQ ID NO: 38 - protein, 14 aa, synthetic construct
WFRQRPGKELEFVA

SEQ ID NO: 39 - protein, 14 aa, synthetic construct
WFRQRPGKEIEFVA

SEQ ID NO: 40 - protein, 14 aa, synthetic construct
WFRQRPGKERELVA

SEQ ID NO: 41 - protein, 14 aa, synthetic construct
WFRQRPGRAREFVA

SEQ ID NO: 42-44 - skipped (3 entries)

SEQ ID NO: 45 - protein, 39 aa, synthetic construct
YADSVKGRFTISRDNAKNTVYLQMNSLKPEDTAVYYCAA

SEQ ID NO: 46 - protein, 39 aa, synthetic construct
YNDSVKGRFTISRDNAKNTVYLQMNSLKPEDTAVYYCAA

SEQ ID NO: 47 - protein, 39 aa, synthetic construct
YQDSVKGRFTISRDNAKNTVYLQMNSLKPEDTAVYYCAA

SEQ ID NO: 48 - protein, 39 aa, synthetic construct
YTDSVKGRFTISRDNAKNTVYLQMNSLKPEDTAVYYCAA

SEQ ID NO: 49 - protein, 39 aa, synthetic construct
YSDSVKGRFTISRDNAKNTVYLQMNSLKPEDTAVYYCAA

SEQ ID NO: 50 - protein, 39 aa, synthetic construct
YVDSVKGRFTISRDNAKNTVYLQMNSLKPEDTAVYYCAA

SEQ ID NO: 51 - skipped

SEQ ID NO: 52 - protein, 39 aa, synthetic construct
YADSVKGRFTISRDNAKSTVYLQMNSLKPEDTAVYYCAA

SEQ ID NO: 53 - protein, 39 aa, synthetic construct
YADSVKGRFTISRDNAKETVYLQMNSLKPEDTAVYYCAA

SEQ ID NO: 54 - protein, 39 aa, synthetic construct
YADSVKGRFTISRDNAKQTVYLQMNSLKPEDTAVYYCAA

SEQ ID NO: 55 - protein, 39 aa, synthetic construct
YADSVKGRFTISRDNAKDTVYLQMNSLKPEDTAVYYCAA

SEQ ID NO: 56 - protein, 39 aa, synthetic construct
YADSVKGRFTISRDNAKNTVLLQMNSLKPEDTAVYYCAA

SEQ ID NO: 57 - protein, 39 aa, synthetic construct
YADSVKGRFTISRDNAKNTVVLQMNSLKPEDTAVYYCAA

SEQ ID NO: 58 - protein, 39 aa, synthetic construct
YADSVKGRFTISRDNAKNTVALQMNSLKPEDTAVYYCAA

SEQ ID NO: 59 - protein, 39 aa, synthetic construct
YADSVKGRFTISRDNAKNTVFLQMNSLKPEDTAVYYCAA

SEQ ID NO: 60 - protein, 39 aa, synthetic construct
YADSVKGRFTISRDNAKNTVWLQMNSLKPEDTAVYYCAA

SEQ ID NO: 61 - protein, 39 aa, synthetic construct
YADSVKGRFTISRDNAKNTVYLQMNNLKPEDTAVYYCAA

SEQ ID NO: 62 - protein, 39 aa, synthetic construct
YADSVKGRFTISRDNAKNTVYLQMNTLKPEDTAVYYCAA

SEQ ID NO: 63 - protein, 39 aa, synthetic construct
YADSVKGRFTISRDNAKNTVYLQMNQLKPEDTAVYYCAA

SEQ ID NO: 64 - skipped

SEQ ID NO: 65 - protein, 39 aa, synthetic construct
YADSVKGRFTISRDNAKNTVYLQMNSLKPEDTAAYYCAA

SEQ ID NO: 66 - skipped

SEQ ID NO: 67 - protein, 39 aa, synthetic construct
YADSVKGRFTISRDNAKNTVYLQMNSLKPEDTAIYYCAA

SEQ ID NO: 68 - protein, 39 aa, synthetic construct
YADSVKGRFTISRDNAKNTVYLQMNSLKPEDTALYYCAA

SEQ ID NO: 69 - protein, 39 aa, synthetic construct
YTDSVKGRFTISRDNAKNTVFLQMQSLKPEDTAIYYCAA

SEQ ID NO: 70 - protein, 39 aa, synthetic construct
YTDSVKGRFTISRDNAKNTVYLQMQSLKPEDTAVYYCAA

SEQ ID NO: 71 - protein, 11 aa, Lama glama
WGQGTQVTVSS

SEQ ID NO: 72 - protein, 126 aa, synthetic construct
QVQLQESGGGSVQAGGSLRLSCVASGRTLSDYTMGWFRQPPGKAREFVAAISWSGAYTKYADSVKGRFTISRDNAKNTVYLQMNSLKPEDTAVYYCAAGPTGLLSKKATPADYDYWGQGTQVTVSS

SEQ ID NO: 73 - protein, 126 aa, synthetic construct
QVQLQESGGGSVQAGGSLRLSCVASGRTLSDYTMGWFRQPPGKAREFVAAISWSGAYTYYADSVKGRFTISRDNAKNTVYLQMNSLKPEDTAVYYCAAGPTGLLSKKATPADYDYWGQGTQVTVSS

SEQ ID NO: 74 - protein, 126 aa, synthetic construct
QVQLQESGGGSVQAGGSLTLSCVASGRTLSDYTMGWFRQPPGKAREFVAAISWSGAYTYYADSVKGRFTISRDNAKNTVYLQMNSLKPEDTAVYYCAAGPTGLLSKKATPADYDYWGQGTQVTVSS

SEQ ID NO: 75 - protein, 126 aa, synthetic construct
QVQLQESGGGSVQAGGSLRLSCTASGRTLSDYTMGWFRQPPGKAREFVAAISWSGAYTYYADSVKGRFTISRDNAKNTVYLQMNSLKPEDTAVYYCAAGPTGLLSKKATPADYDYWGQGTQVTVSS

SEQ ID NO: 76 - protein, 126 aa, synthetic construct
QVQLQESGGGSVQAGGSLRLSCVASGRTLSDYTMGWFRQRPGKAREFVAAISWSGAYTYYADSVKGRFTISRDNAKNTVYLQMNSLKPEDTAVYYCAAGPTGLLSKKATPADYDYWGQGTQVTVSS

SEQ ID NO: 77 - protein, 126 aa, synthetic construct
QVQLQESGGGSVQAGGSLTLSCTASGRTLSDYTMGWFRQPPGKAREFVAAISWSGAYTYYADSVKGRFTISRDNAKNTVYLQMNSLKPEDTAVYYCAAGPTGLLSKKATPADYDYWGQGTQVTVSS

SEQ ID NO: 78 - protein, 126 aa, synthetic construct
QVQLQESGGGSVQAGGSLTLSCTASGRTLSDYTMGWFRQRPGKAREFVAAISWSGAYTYYADSVKGRFTISRDNAKNTVYLQMNSLKPEDTAVYYCAAGPTGLLSKKATPADYDYWGQGTQVTVSS

SEQ ID NO: 79 - skipped

SEQ ID NO: 80 - protein, 126 aa, synthetic construct
QVQLQQSGGGSVQAGGSLRLSCTISGRTLSDYTMGWFRQRPGKEREFVAAISWSGAYTKYADSVKGRFTISRDNAKNTVYLQMNSLKPEDTAVYYCAAGPTGLLSKKATPADYDYWGQGTQVTVSS

SEQ ID NO: 81 - protein, 126 aa, synthetic construct
QVQLQESGGGSVQAGGSLRLSCTISGRTLSDYTMGWFRQRPGKEREFVAAISWSGAYTKYADSVKGRFTISRDNAKNTVYLQMNSLKPEDTAVYYCAAGPTGLLSKKATPADYDYWGQGTQVTVSS

SEQ ID NO: 82 - protein, 126 aa, synthetic construct
QVQLQQSGGGSVQAGGSLRLSCTVSGRTLSDYTMGWFRQRPGKEREFVAAISWSGAYTKYADSVKGRFTISRDNAKNTVYLQMNSLKPEDTAVYYCAAGPTGLLSKKATPADYDYWGQGTQVTVSS

SEQ ID NO: 83 - protein, 126 aa, synthetic construct
QVQLQQSGGGSVQAGGSLRLSCTISGRTLSDYTMGWFRQPPGKEREFVAAISWSGAYTKYADSVKGRFTISRDNAKNTVYLQMNSLKPEDTAVYYCAAGPTGLLSKKATPADYDYWGQGTQVTVSS

SEQ ID NO: 84 - protein, 126 aa, synthetic construct
QVQLQQSGGGSVQAGGSLRLSCTISGRTLSDYTMGWFRQRPGKAREFVAAISWSGAYTKYADSVKGRFTISRDNAKNTVYLQMNSLKPEDTAVYYCAAGPTGLLSKKATPADYDYWGQGTQVTVSS

SEQ ID NO: 85 - protein, 126 aa, synthetic construct
QVQLQESGGGSVQAGGSLRLSCTISGRTLSDYTMGWFRQRPGKAREFVAAISWSGAYTKYADSVKGRFTISRDNAKNTVYLQMNSLKPEDTAVYYCAAGPTGLLSKKATPADYDYWGQGTQVTVSS

SEQ ID NO: 86 - protein, 126 aa, synthetic construct
QVQLQQSGGGSVQAGGSLRLSCTVSGRTLSDYTMGWFRQRPGKAREFVAAISWSGAYTKYADSVKGRFTISRDNAKNTVYLQMNSLKPEDTAVYYCAAGPTGLLSKKATPADYDYWGQGTQVTVSS

SEQ ID NO: 87 - protein, 126 aa, synthetic construct
QVQLQQSGGGSVQAGGSLRLSCTISGRTLSDYTMGWFRQPPGKAREFVAAISWSGAYTKYADSVKGRFTISRDNAKNTVYLQMNSLKPEDTAVYYCAAGPTGLLSKKATPADYDYWGQGTQVTVSS

SEQ ID NO: 88 - protein, 126 aa, synthetic construct
QVQLQQSGGGSVQAGGSLTLSCTISGRTLSDYTMGWFRQRPGKEREFVAAISWSGAYTKYADSVKGRFTISRDNAKNTVYLQMNSLKPEDTAVYYCAAGPTGLLSKKATPADYDYWGQGTQVTVSS

SEQ ID NO: 89 - protein, 126 aa, synthetic construct
QVQLVQSGGGSVQAGGSLRLSCTISGRTLSDYTMGWFRQRPGKEREFVAAISWSGAYTKYADSVKGRFTISRDNAKNTVYLQMNSLKPEDTAVYYCAAGPTGLLSKKATPADYDYWGQGTQVTVSS

SEQ ID NO: 90 - protein, 126 aa, synthetic construct
QVQLEQSGGGSVQAGGSLRLSCTISGRTLSDYTMGWFRQRPGKEREFVAAISWSGAYTKYADSVKGRFTISRDNAKNTVYLQMNSLKPEDTAVYYCAAGPTGLLSKKATPADYDYWGQGTQVTVSS

SEQ ID NO: 91 - protein, 126 aa, synthetic construct; identical to SEQ ID NO: 81

SEQ ID NO: 92 - protein, 126 aa, synthetic construct
QVQLQQSGGGSVQSGGSLRLSCTISGRTLSDYTMGWFRQRPGKEREFVAAISWSGAYTKYADSVKGRFTISRDNAKNTVYLQMNSLKPEDTAVYYCAAGPTGLLSKKATPADYDYWGQGTQVTVSS

SEQ ID NO: 93 - protein, 126 aa, synthetic construct
QVQLQQSGGGSVQTGGSLRLSCTISGRTLSDYTMGWFRQRPGKEREFVAAISWSGAYTKYADSVKGRFTISRDNAKNTVYLQMNSLKPEDTAVYYCAAGPTGLLSKKATPADYDYWGQGTQVTVSS

SEQ ID NO: 94 - protein, 126 aa, synthetic construct
QVQLQQSGGGSVQAGGSLKLSCTISGRTLSDYTMGWFRQRPGKEREFVAAISWSGAYTKYADSVKGRFTISRDNAKNTVYLQMNSLKPEDTAVYYCAAGPTGLLSKKATPADYDYWGQGTQVTVSS

SEQ ID NO: 95 - protein, 126 aa, synthetic construct
QVQLQQSGGGSVQAGGSLSLSCTISGRTLSDYTMGWFRQRPGKEREFVAAISWSGAYTKYADSVKGRFTISRDNAKNTVYLQMNSLKPEDTAVYYCAAGPTGLLSKKATPADYDYWGQGTQVTVSS

SEQ ID NO: 96 - protein, 126 aa, synthetic construct
QVQLQQSGGGSVQAGGSLRLSCVISGRTLSDYTMGWFRQRPGKEREFVAAISWSGAYTKYADSVKGRFTISRDNAKNTVYLQMNSLKPEDTAVYYCAAGPTGLLSKKATPADYDYWGQGTQVTVSS

SEQ ID NO: 97 - protein, 126 aa, synthetic construct
QVQLQQSGGGSVQAGGSLRLSCSISGRTLSDYTMGWFRQRPGKEREFVAAISWSGAYTKYADSVKGRFTISRDNAKNTVYLQMNSLKPEDTAVYYCAAGPTGLLSKKATPADYDYWGQGTQVTVSS

SEQ ID NO: 98 - protein, 126 aa, synthetic construct
QVQLQQSGGGSVQAGGSLRLSCAISGRTLSDYTMGWFRQRPGKEREFVAAISWSGAYTKYADSVKGRFTISRDNAKNTVYLQMNSLKPEDTAIYYCAAGPTGLLSKKATPADYDYWGQGTQVTVSS

SEQ ID NO: 99 - protein, 126 aa, synthetic construct
QVQLQQSGGGSVQAGGSLRLSCTSSGRTLSDYTMGWFRQRPGKEREFVAAISWSGAYTKYADSVKGRFTISRDNAKNTVYLQMNSLKPEDTAVYYCAAGPTGLLSKKATPADYDYWGQGTQVTVSS

SEQ ID NO: 100 - protein, 126 aa, synthetic construct; identical to SEQ ID NO: 82

SEQ ID NO: 101 - protein, 126 aa, synthetic construct
QVQLQQSGGGSVQAGGSLRLSCTISGRTLSDYTMGWFRQTPGKEREFVAAISWSGAYTKYADSVKGRFTISRDNAKNTVYLQMNSLKPEDTAVYYCAAGPTGLLSKKATPADYDYWGQGTQVTVSS

SEQ ID NO: 102 - protein, 126 aa, synthetic construct
QVQLQQSGGGSVQAGGSLRLSCTISGRTLSDYTMGWFRQIPGKEREFVAAISWSGAYTKYADSVKGRFTISRDNAKNTVYLQMNSLKPEDTAVYYCAAGPTGLLSKKATPADYDYWGQGTQVTVSS

SEQ ID NO: 103 - protein, 126 aa, synthetic construct
QVQLQQSGGGSVQAGGSLRLSCTISGRTLSDYTMGWFRQKPGKEREFVAAISWSGAYTKYADSVKGRFTISRDNAKNTVYLQMNSLKPEDTAVYYCAAGPTGLLSKKATPADYDYWGQGTQVTVSS

SEQ ID NO: 104 - protein, 126 aa, synthetic construct
QVQLQQSGGGSVQAGGSLRLSCTISGRTLSDYTMGWFRQAPGKEREFVAAISWSGAYTKYADSVKGRFTISRDNAKNTVYLQMNSLKPEDTAIYYCAAGPTGLLSKKATPADYDYWGQGTQVTVSS

SEQ ID NO: 105 - protein, 126 aa, synthetic construct
QVQLQQSGGGSVQAGGSLRLSCTISGRTLSDYTMGWFRQRPGGEREFVAAISWSGAYTKYADSVKGRFTISRDNAKNTVYLQMNSLKPEDTAVYYCAAGPTGLLSKKATPADYDYWGQGTQVTVSS

SEQ ID NO: 106 - protein, 126 aa, synthetic construct
QVQLQQSGGGSVQAGGSLRLSCTISGRTLSDYTMGWFRQRPGQEREFVAAISWSGAYTKYADSVKGRFTISRDNAKNTVYLQMNSLKPEDTAVYYCAAGPTGLLSKKATPADYDYWGQGTQVTVSS

SEQ ID NO: 107 - protein, 126 aa, synthetic construct
QVQLQQSGGGSVQAGGSLRLSCTISGRTLSDYTMGWFRQRPGREREFVAAISWSGAYTKYADSVKGRFTISRDNAKNTVYLQMNSLKPEDTAVYYCAAGPTGLLSKKATPADYDYWGQGTQVTVSS

SEQ ID NO: 108 - protein, 126 aa, synthetic construct
QVQLQQSGGGSVQAGGSLRLSCTISGRTLSDYTMGWFRQRPGKQREFVAAISWSGAYTKYADSVKGRFTISRDNAKNTVYLQMNSLKPEDTAVYYCAAGPTGLLSKKATPADYDYWGQGTQVTVSS

SEQ ID NO: 109 - protein, 126 aa, synthetic construct; identical to SEQ ID NO: 84

SEQ ID NO: 110 - protein, 126 aa, synthetic construct
QVQLQQSGGGSVQAGGSLRLSCTISGRTLSDYTMGWFRQRPGKDREFVAAISWSGAYTKYADSVKGRFTISRDNAKNTVYLQMNSLKPEDTAVYYCAAGPTGLLSKKATPADYDYWGQGTQVTVSS

SEQ ID NO: 111 - protein, 126 aa, synthetic construct
QVQLQQSGGGSVQAGGSLRLSCTISGRTLSDYTMGWFRQRPGKGREFVAAISWSGAYTKYADSVKGRFTISRDNAKNTVYLQMNSLKPEDTAVYYCAAGPTGLLSKKATPADYDYWGQGTQVTVSS

SEQ ID NO: 112 - protein, 126 aa, synthetic construct
QVQLQQSGGGSVQAGGSLRLSCTISGRTLSDYTMGWFRQRPGKELEFVAAISWSGAYTKYADSVKGRFTISRDNAKNTVYLQMNSLKPEDTAVYYCAAGPTGLLSKKATPADYDYWGQGTQVTVSS

SEQ ID NO: 113 - protein, 126 aa, synthetic construct
QVQLQQSGGGSVQAGGSLRLSCTISGRTLSDYTMGWFRQRPGKEIEFVAAISWSGAYTKYADSVKGRFTISRDNAKNTVYLQMNSLKPEDTAVYYCAAGPTGLLSKKATPADYDYWGQGTQVTVSS

SEQ ID NO: 114 - protein, 126 aa, synthetic construct
QVQLQQSGGGSVQAGGSLRLSCTISGRTLSDYTMGWFRQRPGKERELVAAISWSGAYTKYADSVKGRFTISRDNAKNTVYLQMNSLKPEDTAIYYCAAGPTGLLSKKATPADYDYWGQGTQVTVSS

SEQ ID NO: 115-117 - skipped (3 entries)

SEQ ID NO: 118 - protein, 126 aa, synthetic construct
QVQLQQSGGGSVQAGGSLRLSCTISGRTLSDYTMGWFRQRPGKEREFVAAISWSGAYTKYNDSVKGRFTISRDNAKNTVYLQMNSLKPEDTAVYYCAAGPTGLLSKKATPADYDYWGQGTQVTVSS

SEQ ID NO: 119 - protein, 126 aa, synthetic construct
QVQLQQSGGGSVQAGGSLRLSCTISGRTLSDYTMGWFRQRPGKEREFVAAISWSGAYTKYQDSVKGRFTISRDNAKNTVYLQMNSLKPEDTAVYYCAAGPTGLLSKKATPADYDYWGQGTQVTVSS

SEQ ID NO: 120 - protein, 126 aa, synthetic construct
QVQLQQSGGGSVQAGGSLRLSCTISGRTLSDYTMGWFRQRPGKEREFVAAISWSGAYTKYTDSVKGRFTISRDNAKNTVYLQMNSLKPEDTAVYYCAAGPTGLLSKKATPADYDYWGQGTQVTVSS

SEQ ID NO: 121 - protein, 126 aa, synthetic construct
QVQLQQSGGGSVQAGGSLRLSCTISGRTLSDYTMGWFRQRPGKEREFVAAISWSGAYTKYSDSVKGRFTISRDNAKNTVYLQMNSLKPEDTAVYYCAAGPTGLLSKKATPADYDYWGQGTQVTVSS

SEQ ID NO: 122 - protein, 126 aa, synthetic construct
QVQLQQSGGGSVQAGGSLRLSCTISGRTLSDYTMGWFRQRPGKEREFVAAISWSGAYTKYVDSVKGRFTISRDNAKNTVYLQMNSLKPEDTAVYYCAAGPTGLLSKKATPADYDYWGQGTQVTVSS

SEQ ID NO: 123 - skipped

SEQ ID NO: 124 - protein, 126 aa, synthetic construct
QVQLQQSGGGSVQAGGSLRLSCTISGRTLSDYTMGWFRQRPGKEREFVAAISWSGAYTKYADSVKGRFTISRDNAKSTVYLQMNSLKPEDTAVYYCAAGPTGLLSKKATPADYDYWGQGTQVTVSS

SEQ ID NO: 125 - protein, 126 aa, synthetic construct
QVQLQQSGGGSVQAGGSLRLSCTISGRTLSDYTMGWFRQRPGKEREFVAAISWSGAYTKYADSVKGRFTISRDNAKETVYLQMNSLKPEDTAVYYCAAGPTGLLSKKATPADYDYWGQGTQVTVSS

SEQ ID NO: 126 - protein, 126 aa, synthetic construct
QVQLQQSGGGSVQAGGSLRLSCTISGRTLSDYTMGWFRQRPGKEREFVAAISWSGAYTKYADSVKGRFTISRDNAKQTVYLQMNSLKPEDTAVYYCAAGPTGLLSKKATPADYDYWGQGTQVTVSS

SEQ ID NO: 127 - protein, 126 aa, synthetic construct
QVQLQQSGGGSVQAGGSLRLSCTISGRTLSDYTMGWFRQRPGKEREFVAAISWSGAYTKYADSVKGRFTISRDNAKDTVYLQMNSLKPEDTAVYYCAAGPTGLLSKKATPADYDYWGQGTQVTVSS

SEQ ID NO: 128 - protein, 126 aa, synthetic construct
QVQLQQSGGGSVQAGGSLRLSCTISGRTLSDYTMGWFRQRPGKEREFVAAISWSGAYTKYADSVKGRFTISRDNAKNTVLLQMNSLKPEDTAVYYCAAGPTGLLSKKATPADYDYWGQGTQVTVSS

SEQ ID NO: 129 - protein, 126 aa, synthetic construct
QVQLQQSGGGSVQAGGSLRLSCTISGRTLSDYTMGWFRQRPGKEREFVAAISWSGAYTKYADSVKGRFTISRDNAKNTVVLQMNSLKPEDTAVYYCAAGPTGLLSKKATPADYDYWGQGTQVTVSS

SEQ ID NO: 130 - protein, 126 aa, synthetic construct
QVQLQQSGGGSVQAGGSLRLSCTISGRTLSDYTMGWFRQRPGKEREFVAAISWSGAYTKYADSVKGRFTISRDNAKNTVALQMNSLKPEDTAVYYCAAGPTGLLSKKATPADYDYWGQGTQVTVSS

SEQ ID NO: 131 - protein, 126 aa, synthetic construct
QVQLQQSGGGSVQAGGSLRLSCTISGRTLSDYTMGWFRQRPGKEREFVAAISWSGAYTKYADSVKGRFTISRDNAKNTVFLQMNSLKPEDTAVYYCAAGPTGLLSKKATPADYDYWGQGTQVTVSS

SEQ ID NO: 132 - protein, 126 aa, synthetic construct
QVQLQQSGGGSVQAGGSLRLSCTISGRTLSDYTMGWFRQRPGKEREFVAAISWSGAYTKYADSVKGRFTISRDNAKNTVWLQMNSLKPEDTAVYYCAAGPTGLLSKKATPADYDYWGQGTQVTVSS

SEQ ID NO: 133 - protein, 126 aa, synthetic construct
QVQLQQSGGGSVQAGGSLRLSCTISGRTLSDYTMGWFRQRPGKEREFVAAISWSGAYTKYADSVKGRFTISRDNAKNTVYLQMNNLKPEDTAVYYCAAGPTGLLSKKATPADYDYWGQGTQVTVSS

SEQ ID NO: 134 - protein, 126 aa, synthetic construct
QVQLQQSGGGSVQAGGSLRLSCTISGRTLSDYTMGWFRQRPGKEREFVAAISWSGAYTKYADSVKGRFTISRDNAKNTVYLQMNTLKPEDTAVYYCAAGPTGLLSKKATPADYDYWGQGTQVTVSS

SEQ ID NO: 135 - protein, 126 aa, synthetic construct
QVQLQQSGGGSVQAGGSLRLSCTISGRTLSDYTMGWFRQRPGKEREFVAAISWSGAYTKYADSVKGRFTISRDNAKNTVYLQMNQLKPEDTAVYYCAAGPTGLLSKKATPADYDYWGQGTQVTVSS

SEQ ID NO: 136 - skipped

SEQ ID NO: 137 - protein, 126 aa, synthetic construct
QVQLQQSGGGSVQAGGSLRLSCTISGRTLSDYTMGWFRQRPGKEREFVAAISWSGAYTKYADSVKGRFTISRDNAKNTVYLQMNSLKPEDTAAYYCAAGPTGLLSKKATPADYDYWGQGTQVTVSS

SEQ ID NO: 138 - skipped

SEQ ID NO: 139 - protein, 126 aa, synthetic construct
QVQLQQSGGGSVQAGGSLRLSCTISGRTLSDYTMGWFRQRPGKEREFVAAISWSGAYTKYADSVKGRFTISRDNAKNTVYLQMNSLKPEDTAIYYCAAGPTGLLSKKATPADYDYWGQGTQVTVSS

SEQ ID NO: 140 - protein, 126 aa, synthetic construct
QVQLQQSGGGSVQAGGSLRLSCTISGRTLSDYTMGWFRQRPGKEREFVAAISWSGAYTKYADSVKGRFTISRDNAKNTVYLQMNSLKPEDTALYYCAAGPTGLLSKKATPADYDYWGQGTQVTVSS

SEQ ID NO: 141 - protein, 126 aa, synthetic construct; identical to SEQ ID NO: 98

SEQ ID NO: 142 - protein, 126 aa, synthetic construct; identical to SEQ ID NO: 104

SEQ ID NO: 143 - protein, 126 aa, synthetic construct; identical to SEQ ID NO: 114

SEQ ID NO: 144 - protein, 126 aa, synthetic construct
QVQLQQSGGGSVQAGGSLRLSCTSSGRTLSDFTMAWFRQRPGRAREFVAAISWSGAYTYYTDSVKGRFTISRDNAKNTVFLQMQSLKPEDTAIYYCAAGPTGLLSRKTTPADYQYWGQGTQVTVSS

SEQ ID NO: 145 - protein, 126 aa, synthetic construct
QVQLVESGGGSVQAGGSLSLSCTISGRTLSDFTMAWFRQRPGKEREFVAAISWSGAYTYYTDSVKGRFTISRDNAKNTVYLQMQSLKPEDTAVYYCAAGPTGLLSRKTTPADYQYWGQGTQVTVSS

SEQ ID NO: 146 - protein, 126 aa, synthetic construct
QVQLQQSGGGSVQAGGSLRLSCTISGRTLSDFTMAWFRQRPGKEREFVAAISWSGAYTYYADSVKGRFTISRDNAKNTVYLQMNSLKPEDTAVYYCAAGPTGLLSRKTTPADYQYWGQGTQVTVSS

SEQ ID NO: 147 - protein, 126 aa, synthetic construct
QVQLQQSGGGSVQAGGSLRLSCTISGRTLSDFTMAWFRQRPGKEREFVAAVSWSGAYTKYADSVKGRFTISRDNAKNTVYLQMNSLKPEDTAVYYCAAGPTGLLSKKATPPDYDYWGQGTQVTVSS

SEQ ID NO: 148 - protein, 126 aa, synthetic construct
QVQLQQSGGGSVQAGGSLRLSCTISGRTLSDFTMGWFRQRPGKEREFVAAISWSGAYTKYADSVKGRFTISRDNAKNTVYLQMNSLKPEDTAVYYCAAGPTGLLSKKTTPADYDYWGQGTQVTVSS

SEQ ID NO: 149 - protein, 126 aa, synthetic construct
QVQLQQSGGGSVQAGGSLTLSCTVSGRTLSDFTMGWFRQRPGKELEFVAAISWSGAYTKYADSVKGRFTISRDNAKNTVWLQMNSLKPEDTAVYYCAAGPTGPLSKKTTPADYDYWGQGTQVTVSS

SEQ ID NO: 150 - protein, 126 aa, synthetic construct
QVQLQQSGGGSVQAGGSLRLSCTSSGRTLSDFTMGWFRQRPGKEREFVAAISWSGAYTKYADSVKGRFTISRDNAKNTVWLQMNSLKPEDTAVYYCAAGPTGLLSKKTTPADYDYWGQGTQVTVSS

SEQ ID NO: 151 - protein, 126 aa, synthetic construct
QVQLQQSGGGSVQAGGSLRLSCTVSGRTLSDFTMGWFRQRPGKEREFVAAISWSGAYTKYADSVKGRFTISRDNAKNTVFLQMNSLKPEDTALYYCAAGPTGLLSKKTTPADYDYWGQGTQVTVSS

SEQ ID NO: 152 - protein, 126 aa, synthetic construct
QVQLQESGGGLVQPGGSLRLSCAASGRTLSDYTMGWFRQAPGKQREFVAAISWSGAYTKYTDSVKGRFTISRDNAKTTVYLQMNSLKPEDTAVYYCAAGPTGLLSKKATPADYDYWGQGTQVTVSS

SEQ ID NO: 153 - protein, 126 aa, synthetic construct
EVQLVESGGGLVQAGGSLRLSCAASGRTLSDYTMGWFRQAPGKEREFVVAISWSGAYTKYADSVKGRFTISRDNAKNTMYLQMNSLKPEDTAVYYCAAGPTGLLSKKATPADYDYWGQGTQVTVSS

SEQ ID NO: 154 - protein, 128 aa, synthetic construct
VDQLQESGGGSVQAGEALRLSCVGSGYTSINPYMAWFRQAPGKEREGVAAISSGGVYTYYADSVKGRFTITRDNVKNTMYLQMPSLKPEDSAKYYCAADFRRGGNWNVDPFRYDYQHWGQGTQVTVSS

SEQ ID NO: 155 - protein, 128 aa, synthetic construct
QVQLQESGGGLVQPGGSLRLSCAASGRTSINPYMAWFRQAPGKQREFVAAISSGGVYTYYTDSVKGRFTISRDNAKTTVYLQMNSLKPEDTAVYYCAADFRRGGNWNVDPFRYDYQYWGQGTQVTVSS

SEQ ID NO: 156 - protein, 128 aa, synthetic construct
QVQLQQSGGGSVQAGGSLRLSCTISGRTSINPYMAWFRQRPGKEREFVAAISSGGVYTYYADSVKGRFTISRDNAKNTVYLQMNSLKPEDTAVYYCAADFRRGGNWNVDPFRYDYDYWGQGTQVTVSS

SEQ ID NO: 157 - protein, 127 aa, Lama glama
EVQLVESGGGLVQAGGSLRLSCAASGRTFSSYAMGWFRQAPGKEREFVVAINWSSGSTYYADSVKGRFTISRDNAKNTMYLQMNSLKPEDTAVYYCAAGYQINSGNYNFKDYEYDYWGQGTQVTVSS

SEQ ID NO: 158 - protein, 127 aa, synthetic construct
QVQLQQSGGGSVQAGGSLRLSCTISGRTFSSYAMGWFRQRPGKEREFVAAINWSSGSTYYADSVKGRFTISRDNAKNTVYLQMNSLKPEDTAVYYCAAGYQINSGNYNFKDYEYDYWGQGTQVTVSS

SEQ ID NO: 159 - protein, 58 aa, synthetic construct
VDAKFDKEAQEAFYEILHLPNLTEEQRNAFIQSLKDDPSGSKAILAEAKKVNDAQAPK

SEQ ID NO: 160 - protein, 58 aa, synthetic construct
VDAKFDKEAYRALAEIARLPNLTEEQRAAFIQSLKDDPSGSKAILAEAKKVNDAQAPK

SEQ ID NO: 161 - protein, 200 aa, synthetic construct
  SIGNAL 1..4
AQGTQVQLQQSGGGSVQAGGSLRLSCTISGRTLSDYTMGWFRQRPGKEREFVAAISWSGAYTKYADSVKGRFTISRDNAKNTVYLQMNSLKPEDTAVYYCAAGPTGLLSKKATPADYDYWGQGTQVTVSSQASVDAKFDKEAYRALAEIARLPNLTEEQRAAFIQSLKDDPSGSKAILAEAKKVNDAQAPKGSHHHHHHC

SEQ ID NO: 162 - protein, 195 aa, synthetic construct
QVQLQQSGGGSVQAGGSLRLSCTISGRTLSDYTMGWFRQRPGKEREFVAAISWSGAYTKYADSVKGRFTISRDNAKNTVYLQMNSLKPEDTAVYYCAAGPTGLLSKKATPADYDYWGQGTQVTVSSQASVDAKFDKEAYRALAEIARLPNLTEEQRAAFIQSLKDDPSGSKAILAEAKKVNDAQAPKGSHHHHHH

SEQ ID NO: 163 - protein, 195 aa, synthetic construct
QVQLQESGGGLVQPGGSLRLSCAASGRTLSDYTMGWFRQAPGKQREFVAAISWSGAYTKYTDSVKGRFTISRDNAKTTVYLQMNSLKPEDTAVYYCAAGPTGLLSKKATPADYDYWGQGTQVTVSSQASVDAKFDKEAYRALAEIARLPNLTEEQRAAFIQSLKDDPSGSKAILAEAKKVNDAQAPKGSHHHHHH

SEQ ID NO: 164 - protein, 195 aa, synthetic construct
EVQLVESGGGLVQAGGSLRLSCAASGRTLSDYTMGWFRQAPGKEREFVVAISWSGAYTKYADSVKGRFTISRDNAKNTMYLQMNSLKPEDTAVYYCAAGPTGLLSKKATPADYDYWGQGTQVTVSSQASVDAKFDKEAYRALAEIARLPNLTEEQRAAFIQSLKDDPSGSKAILAEAKKVNDAQAPKGSHHHHHH

SEQ ID NO: 165 - protein, 197 aa, synthetic construct
VDQLQESGGGSVQAGEALRLSCVGSGYTSINPYMAWFRQAPGKEREGVAAISSGGVYTYYADSVKGRFTITRDNVKNTMYLQMPSLKPEDSAKYYCAADFRRGGNWNVDPFRYDYQHWGQGTQVTVSSQASVDAKFDKEAYRALAEIARLPNLTEEQRAAFIQSLKDDPSGSKAILAEAKKVNDAQAPKGSHHHHHH

SEQ ID NO: 166 - protein, 197 aa, synthetic construct
QVQLQESGGGLVQPGGSLRLSCAASGRTSINPYMAWFRQAPGKQREFVAAISSGGVYTYYTDSVKGRFTISRDNAKTTVYLQMNSLKPEDTAVYYCAADFRRGGNWNVDPFRYDYQYWGQGTQVTVSSQASVDAKFDKEAYRALAEIARLPNLTEEQRAAFIQSLKDDPSGSKAILAEAKKVNDAQAPKGSHHHHHH

SEQ ID NO: 167 - protein, 197 aa, synthetic construct
QVQLQQSGGGSVQAGGSLRLSCTISGRTSINPYMAWFRQRPGKEREFVAAISSGGVYTYYADSVKGRFTISRDNAKNTVYLQMNSLKPEDTAVYYCAADFRRGGNWNVDPFRYDYDYWGQGTQVTVSSQASVDAKFDKEAYRALAEIARLPNLTEEQRAAFIQSLKDDPSGSKAILAEAKKVNDAQAPKGSHHHHHH

SEQ ID NO: 168 - protein, 196 aa, synthetic construct
EVQLVESGGGLVQAGGSLRLSCAASGRTFSSYAMGWFRQAPGKEREFVVAINWSSGSTYYADSVKGRFTISRDNAKNTMYLQMNSLKPEDTAVYYCAAGYQINSGNYNFKDYEYDYWGQGTQVTVSSQASVDAKFDKEAYRALAEIARLPNLTEEQRAAFIQSLKDDPSGSKAILAEAKKVNDAQAPKGSHHHHHH

SEQ ID NO: 169 - protein, 196 aa, synthetic construct
QVQLQQSGGGSVQAGGSLRLSCTISGRTFSSYAMGWFRQRPGKEREFVAAINWSSGSTYYADSVKGRFTISRDNAKNTVYLQMNSLKPEDTAVYYCAAGYQINSGNYNFKDYEYDYWGQGTQVTVSSQASVDAKFDKEAYRALAEIARLPNLTEEQRAAFIQSLKDDPSGSKAILAEAKKVNDAQAPKGSHHHHHH

SEQ ID NO: 170 - protein, 200 aa, synthetic construct
  SIGNAL 1..4
AQGTQVQLQESGGGSVQAGGSLRLSCVASGRTLSDYTMGWFRQPPGKAREFVAAISWSGAYTKYADSVKGRFTISRDNAKNTVYLQMNSLKPEDTAVYYCAAGPTGLLSKKATPADYDYWGQGTQVTVSSQASVDAKFDKEAQEAFYEILHLPNLTEEQRNAFIQSLKDDPSGSKAILAEAKKVNDAQAPKGSHHHHHHC

SEQ ID NO: 171 - protein, 200 aa, synthetic construct
  SIGNAL 1..4
AQGTQVQLQQSGGGSVQAGGSLRLSCTISGRTLSDYTMGWFRQRPGKEREFVAAISWSGAYTKYADSVKGRFTISRDNAKNTVYLQMNSLKPEDTAVYYCAAGPTGLLSKKATPADYDYWGQGTQVTVSSQASVDAKFDKEAQEAFYEILHLPNLTEEQRNAFIQSLKDDPSGSKAILAEAKKVNDAQAPKGSHHHHHHC

SEQ ID NO: 172 - protein, 202 aa, synthetic construct
  SIGNAL 1..4
AQGTQVQLQESGGGLVQPGGSLRLSCAASGRTSINPYMAWFRQAPGKQREFVAAISSGGVYTYYTDSVKGRFTISRDNAKTTVYLQMNSLKPEDTAVYYCAADFRRGGNWNVDPFRYDYQYWGQGTQVTVSSQASVDAKFDKEAQEAFYEILHLPNLTEEQRNAFIQSLKDDPSGSKAILAEAKKVNDAQAPKGSHHHHHHC

SEQ ID NO: 173 - protein, 202 aa, synthetic construct
  SIGNAL 1..4
AQGTQVQLQQSGGGSVQAGGSLRLSCTISGRTSINPYMAWFRQRPGKEREFVAAISSGGVYTYYADSVKGRFTISRDNAKNTVYLQMNSLKPEDTAVYYCAADFRRGGNWNVDPFRYDYDYWGQGTQVTVSSQASVDAKFDKEAQEAFYEILHLPNLTEEQRNAFIQSLKDDPSGSKAILAEAKKVNDAQAPKGSHHHHHHC

SEQ ID NO: 174 - protein, 197 aa, synthetic construct
EVQLVESGGGLVQAGGSLRLSCAASGRTFSSYAMGWFRQAPGKEREFVVAINWSSGSTYYADSVKGRFTISRDNAKNTMYLQMNSLKPEDTAVYYCAAGYQINSGNYNFKDYEYDYWGQGTQVTVSSQASVDAKFDKEAQEAFYEILHLPNLTEEQRNAFIQSLKDDPSGSKAILAEAKKVNDAQAPKGSHHHHHHC

SEQ ID NO: 175 - protein, 197 aa, synthetic construct
QVQLQQSGGGSVQAGGSLRLSCTISGRTFSSYAMGWFRQRPGKEREFVAAINWSSGSTYYADSVKGRFTISRDNAKNTVYLQMNSLKPEDTAVYYCAAGYQINSGNYNFKDYEYDYWGQGTQVTVSSQASVDAKFDKEAQEAFYEILHLPNLTEEQRNAFIQSLKDDPSGSKAILAEAKKVNDAQAPKGSHHHHHHC

SEQ ID NO: 176 - protein, 9 aa, synthetic construct
RTLSDYTMG

SEQ ID NO: 177 - protein, 9 aa, synthetic construct
RTLSDFTMA

SEQ ID NO: 178 - protein, 9 aa, synthetic construct
RTLSDFTMA

SEQ ID NO: 179 - protein, 9 aa, synthetic construct
RTLSDFTMG

SEQ ID NO: 180 - protein, 10 aa, synthetic construct
AISWSGAYTK

SEQ ID NO: 181 - protein, 10 aa, synthetic construct
AISWSGAYTY

SEQ ID NO: 182 - protein, 10 aa, synthetic construct
AVSWSGAYTK

SEQ ID NO: 183 - protein, 10 aa, synthetic construct
AISWSGAYTK

SEQ ID NO: 184 - protein, 17 aa, synthetic construct
GPTGLLSKKATPADYDY

SEQ ID NO: 185 - protein, 17 aa, synthetic construct
GPTGLLSRKTTPADYQY

SEQ ID NO: 186 - protein, 17 aa, synthetic construct
GPTGLLSKKATPPDYDY

SEQ ID NO: 187 - protein, 17 aa, synthetic construct
GPTGLLSKKTTPADYDY

SEQ ID NO: 188 - protein, 17 aa, synthetic construct
GPTGPLSKKTTPADYDY

SEQ ID NO: 189 - protein, 17 aa, synthetic construct
GPTGLLSKKTTPADYDY

SEQ ID NO: 190 - protein, 26 aa, synthetic construct
QVQLQQSGGGSVQAGGSLTLSCTVSG

SEQ ID NO: 191 - protein, 39 aa, synthetic construct
YADSVKGRFTISRDNAKNTVFLQMNSLKPEDTALYYCAA

SEQ ID NO: 192 - protein, 126 aa, synthetic construct
QVQLQQSGGGSVQAGGSLRLSCTISGRTLHDYTMGWFRQRPGKEREFVAAISWSGAYTKYADSVKGRFTISRDNAKNTVYLQMNSLKPEDTAVYYCAAGPTGLLSKKATPADYDYWGQGTQVTVSS

SEQ ID NO: 193 - protein, 126 aa, synthetic construct
QVQLQQSGGGSVQAGGSLRLSCTISGRTLSDYSMGWFRQRPGKEREFVAAISWSGAYTKYADSVKGRFTISRDNAKNTVYLQMNSLKPEDTAVYYCAAGPTGLLSKKATPADYDYWGQGTQVTVSS

SEQ ID NO: 194 - protein, 26 aa, synthetic construct
EVQLQQSGGGSVQAGGSLRLSCTISG

SEQ ID NO: 195 - protein, 126 aa, synthetic construct
EVQLQQSGGGSVQAGGSLRLSCTISGRTLSDYTMGWFRQRPGKEREFVAAISWSGAYTKYADSVKGRFTISRDNAKNTVYLQMNSLKPEDTAVYYCAAGPTGLLSKKATPADYDYWGQGTQVTVSS